European Patent Application EP 4 389 916 A2, published June 26, 2024. Title: COMPOSITIONS AND METHODS FOR DETECTING GROUP A STREPTOCOCCUS. Applicant: Gen-Probe Incorporated. Application EP. The sequence listing filed with the application follows.

SEQUENCE LISTING (39 sequences)

SEQ ID NO: 1 - DNA, 22 bp, synthetic construct
  misc_feature 1..22: note = Synthetic Oligonucleotide
  source 1..22: mol_type = other DNA
gcaagtagaacgctgagaactg

SEQ ID NO: 2 - DNA, 22 bp, synthetic construct
  misc_feature 1..22: note = Synthetic Oligonucleotide
  source 1..22: mol_type = other DNA
cggttcaaggagttgcgaacgg

SEQ ID NO: 3 - DNA, 20 bp, synthetic construct
  misc_feature 1..20: note = Synthetic Oligonucleotide
  source 1..20: mol_type = other DNA
tatcccccgctatgaggtag

SEQ ID NO: 4 - DNA, 24 bp, synthetic construct
  misc_feature 1..24: note = Synthetic Oligonucleotide
  source 1..24: mol_type = other DNA
gggataactattggaaacgatagc

SEQ ID NO: 5 - DNA, 28 bp, synthetic construct
  misc_feature 1..28: note = Synthetic Oligonucleotide
  source 1..28: mol_type = other DNA
ccgcataagagagactaacgcatgttag

SEQ ID NO: 6 - DNA, 22 bp, synthetic construct
  misc_feature 1..22: note = Synthetic Oligonucleotide
  source 1..22: mol_type = other DNA
gcaggtccatctcatagtggag

SEQ ID NO: 7 - DNA, 18 bp, synthetic construct
  misc_feature 1..18: note = Synthetic Oligonucleotide
  source 1..18: mol_type = other DNA
ttgtaggactgcgacgtg

SEQ ID NO: 8 - DNA, 26 bp, synthetic construct
  misc_feature 1..26: note = Synthetic Oligonucleotide
  misc_feature 8: note = N means A or G or C or T/U, unknown, or other.
  source 1..26: mol_type = other DNA
agaagaantacctgggaaggtaagcc

SEQ ID NO: 9 - DNA, 26 bp, synthetic construct
  misc_feature 1..26: note = Synthetic Oligonucleotide
  source 1..26: mol_type = other DNA
gtactcaggatactgctagggctcaa

SEQ ID NO: 10 - DNA, 25 bp, synthetic construct
  misc_feature 1..25: note = Synthetic Oligonucleotide
  source 1..25: mol_type = other DNA
caggataggtaggagccattgactt

SEQ ID NO: 11 - DNA, 27 bp, synthetic construct
  misc_feature 1..27: note = Synthetic Oligonucleotide
  misc_feature 12: note = N means A or G or C or T/U, or unknown, or other.
  source 1..27: mol_type = other DNA
cgaatgaggcgntgttgggatactacc

SEQ ID NO: 12 - DNA, 27 bp, synthetic construct
  misc_feature 1..27: note = Synthetic Oligonucleotide
  source 1..27: mol_type = other DNA
tcagacactgtctccgatagggataac

SEQ ID NO: 13 - DNA, 24 bp, synthetic construct
  misc_feature 1..24: note = Synthetic Oligonucleotide
  source 1..24: mol_type = other DNA
tcagtagcggtagctttgactgtt

SEQ ID NO: 14 - DNA, 27 bp, synthetic construct
  misc_feature 1..27: note = Synthetic Oligonucleotide
  source 1..27: mol_type = other DNA
cttccctaggattaccatcaccgttag

SEQ ID NO: 15 - DNA, 25 bp, synthetic construct
  misc_feature 1..25: note = Synthetic Oligonucleotide
  source 1..25: mol_type = other DNA
ttgcgggattgtttgctgcaagatc

SEQ ID NO: 16 - DNA, 25 bp, synthetic construct
  misc_feature 1..25: note = Synthetic Oligonucleotide
  source 1..25: mol_type = other DNA
ctaataccgcataagagagactaac

SEQ ID NO: 17 - DNA, 25 bp, synthetic construct
  misc_feature 1..25: note = Synthetic Oligonucleotide
  source 1..25: mol_type = other DNA
ctttacctcaccaactagctaatac

SEQ ID NO: 18 - DNA, 25 bp, synthetic construct
  misc_feature 1..25: note = Synthetic Oligonucleotide
  source 1..25: mol_type = other DNA
agtaatttaaaaggggcaattgctc

SEQ ID NO: 19 - DNA, 22 bp, synthetic construct
  misc_feature 1..22: note = Synthetic Oligonucleotide
  source 1..22: mol_type = other DNA
ccgagcgttgtccggatttatt

SEQ ID NO: 20 - DNA, 25 bp, synthetic construct
  misc_feature 1..25: note = Synthetic Oligonucleotide
  source 1..25: mol_type = other DNA
cttctgcactcaagttctccagttt

SEQ ID NO: 21 - DNA, 30 bp, synthetic construct
  misc_feature 1..30: note = Synthetic Oligonucleotide
  source 1..30: mol_type = other DNA
ccaaagcgtacattggttgagccaatgcct

SEQ ID NO: 22 - DNA, 25 bp, synthetic construct
  misc_feature 1..25: note = Synthetic Oligonucleotide
  source 1..25: mol_type = other DNA
gttgaaactcaaaggaattgacggg

SEQ ID NO: 23 - DNA, 25 bp, synthetic construct
  misc_feature 1..25: note = Synthetic Oligonucleotide
  source 1..25: mol_type = other DNA
aaaactctatctctagagcgggcat

SEQ ID NO: 24 - DNA, 28 bp, synthetic construct
  misc_feature 1..28: note = Synthetic Oligonucleotide
  source 1..28: mol_type = other DNA
ggcccgcacaagcggtggagcatgtggt

SEQ ID NO: 25 - DNA, 28 bp, synthetic construct
  misc_feature 1..28: note = Synthetic Oligonucleotide
  source 1..28: mol_type = other DNA
agtaatttaaaaggggcaattgctccac

SEQ ID NO: 26 - DNA, 29 bp, synthetic construct
  misc_feature 1..29: note = Synthetic Oligonucleotide
  source 1..29: mol_type = other DNA
agtggagcaattgccccttttaaattact

SEQ ID NO: 27 - DNA, 19 bp, synthetic construct
  misc_feature 1..19: note = Synthetic Oligonucleotide
  source 1..19: mol_type = other DNA
ctggtgcttgcaccggttc

SEQ ID NO: 28 - DNA, 30 bp, synthetic construct
  misc_feature 1..30: note = Synthetic Oligonucleotide
  source 1..30: mol_type = other DNA
ccttttaaattactaacatgcgttagtctc

SEQ ID NO: 29 - DNA, 32 bp, synthetic construct
  misc_feature 1..32: note = Synthetic Oligonucleotide
  source 1..32: mol_type = other DNA
tcttatgcggtattagctatcgtttccaatag

SEQ ID NO: 30 - DNA, 17 bp, synthetic construct
  misc_feature 1..17: note = Synthetic Oligonucleotide
  source 1..17: mol_type = other DNA
ggtgcttgcaccggttc

SEQ ID NO: 31 - DNA, 22 bp, synthetic construct
  misc_feature 1..22: note = Synthetic Oligonucleotide
  source 1..22: mol_type = other DNA
ccttctacctccactacactga

SEQ ID NO: 32 - DNA, 26 bp, synthetic construct
  misc_feature 1..26: note = Synthetic Oligonucleotide
  source 1..26: mol_type = other DNA
gtcgagtgtctgtgtagatttcagcc

SEQ ID NO: 33 - DNA, 27 bp, synthetic construct
  misc_feature 1..27: note = Synthetic Oligonucleotide
  source 1..27: mol_type = other DNA
caaacggtacaaatcatccagagtgtc

SEQ ID NO: 34 - DNA, 25 bp, synthetic construct
  misc_feature 1..25: note = Synthetic Oligonucleotide
  source 1..25: mol_type = other DNA
gtcctcaatcaaaccttgtcctacc

SEQ ID NO: 35 - DNA, 28 bp, synthetic construct
  misc_feature 1..28: note = Synthetic Oligonucleotide
  source 1..28: mol_type = other DNA
ggtaacagaaatccttgatgagttgcgg

SEQ ID NO: 36 - DNA, 26 bp, synthetic construct
  misc_feature 1..26: note = Synthetic Oligonucleotide
  source 1..26: mol_type = other DNA
gaggtaagaaatagtagcgagtgcgg

SEQ ID NO: 37 - DNA, 26 bp, synthetic construct
  misc_feature 1..26: note = Synthetic Oligonucleotide
  source 1..26: mol_type = other DNA
ccaatcaataccatattccttatccc

SEQ ID NO: 38 - DNA, 22 bp, synthetic construct
  misc_feature 1..22: note = Synthetic Oligonucleotide
  source 1..22: mol_type = other DNA
cggcaacctcttcagtggtttc

SEQ ID NO: 39 - DNA, 28 bp, synthetic construct
  misc_feature 1..28: note = Synthetic Oligonucleotide
  source 1..28: mol_type = other DNA
ccttgccagtattgagagcattatcagc